European Patent Application EP 4 597 113 A1, published August 6, 2025. Title: 질량 보정을 위한 신규한 내부표준물질. Applicant: 씨젠의료재단. Application KR. The sequence listing filed with the application follows.

SEQUENCE LISTING (7 sequences)

SEQ ID NO: 1 - DNA, 30 bp, synthetic construct
  source 1..30: mol_type = other DNA
aactgcaggatgtcactgtatcgccgtcta

SEQ ID NO: 2 - DNA, 45 bp, synthetic construct
  source 1..45: mol_type = other DNA
ggaattctcagtggtggtggtggtggtgctgcccgttgacgccca

SEQ ID NO: 3 - DNA, 30 bp, synthetic construct; identical to SEQ ID NO: 1
  source 1..30: mol_type = other DNA

SEQ ID NO: 4 - DNA, 33 bp, synthetic construct
  source 1..33: mol_type = other DNA
ggaattctcagtggtgctgcccgttgacgccca

SEQ ID NO: 5 - DNA, 30 bp, synthetic construct; identical to SEQ ID NO: 1
  source 1..30: mol_type = other DNA

SEQ ID NO: 6 - DNA, 51 bp, synthetic construct
  source 1..51: mol_type = other DNA
ggaattctcatttttcgaactgcgggtggctccactgcccgttgacgccca

SEQ ID NO: 7 - protein, 8 aa, synthetic construct
WSHPQFEK